European Patent Application EP 4 748 932 A1, published May 27, 2026. Title: TREATMENT AND/OR PREVENTION OF ATHEROSCLEROSIS. Applicant: Fundación Instituto de Investigación Sanitaria Fundación Jiménez Díaz. The sequence listing filed with the application follows.

SEQUENCE LISTING (1 sequence)

SEQ ID NO: 1 - DNA, 21 bp, synthetic construct
  source 1..21: mol_type = other DNA
aggagtgagattgacttaaat